European Patent Specification EP 3 743 447 B1, published March 27, 2024. Title: B7-H4 Antibodies and Methods of Use Thereof. Applicant: NextCure, Inc. Langermann, Soloman Liu, Linda Flies, Dallas B. The sequence listing filed with the application follows.

SEQUENCE LISTING (131 sequences)

SEQ ID NO: 1 - protein, 282 aa, Homo sapiens
MASLGQILFWSIISIIIILAGAIALIIGFGISGRHSITVTTVASAGNIGEDGILSCTFEPDIKLSDIVIQWLKEGVLGLVHEFKEGKDELSEQDEMFRGRTAVFADQVIVGNASLRLKNVQLTDAGTYKCYIITSKGKGNANLEYKTGAFSMPEVNVDYNASSETLRCEAPRWFPQPTVVWASQVDQGANFSEVSNTSFELNSENVTMKVVSVLYNVTINNTYSCMIENDIAKATGDIKVTESEIKRRSHLQLLNSKASLCVSSFFAISWALLPLSPYLMLK

SEQ ID NO: 2 - protein, 283 aa, Mus musculus
MASLGQIIFWSIINIIIILAGAIALIIGFGISGKHFITVTTFTSAGNIGEDGTLSCTFEPDIKLNGIVIQWLKEGIKGLVHEFKEGKDDLSQQHEMFRGRTAVFADQVVVGNASLRLKNVQLTDAGTYTCYIRTSKGKGNANLEYKTGAFSMPEINVDYNASSESLRCEAPRWFPQPTVAWASQVDQGANFSEVSNTSFELNSENVTMKVVSVLYNVTINNTYSCMIENDIAKATGDIKVTDSEVKRRSQLQLLNSGPSPCVFSSAFVAGWALLSLSCCLMLR

SEQ ID NO: 3 - protein, 107 aa, Mus musculus
DIVMTQSHKFMSTSVGDRVSITCKASQDVRTAVAWYQQKPGQSPKLLIYSTSYRYTGVPDRFTGSGSGTEFTFTISSVQAEDLAVYYCQQYYVTPLTFGAGTKLELK

SEQ ID NO: 4 - protein, 11 aa, Mus musculus
KASQDVRTAVA

SEQ ID NO: 5 - protein, 7 aa, Mus musculus
STSYRYT

SEQ ID NO: 6 - protein, 9 aa, Mus musculus
QQYYVTPLT

SEQ ID NO: 7 - DNA, 321 bp, Mus musculus
gacattgtgatgacccagtctcacaaattcatgtccacatcagtaggagacagggtcagtatcacctgcaaggccagtcaggatgtgagaactgctgtagcctggtatcaacagaaaccaggacaatctcctaaactactgatttactcgacatcctaccggtacactggagtccctgatcgcttcactggcagtggatctgggacggaattcactttcaccatcagcagtgtgcaggctgaagacctggcagtttattactgtcagcaatattatgttactccgctcacgttcggtgctgggaccaagctggagctgaaa

SEQ ID NO: 8 - protein, 117 aa, Mus musculus
EVQLQQSGTVLARPGASVKMSCKASGYTFTSYWMHWIKQRPGQGLEWIGAIYPGNSDTKYNQKFKDKAKLTAVTSASTAYMELSSLTNEDSAVYYCTSTVRNVMDYWGQGTSVTVSS

SEQ ID NO: 9 - protein, 5 aa, Mus musculus
SYWMH

SEQ ID NO: 10 - protein, 18 aa, Mus musculus
AIYPGNSDTKYNQKFKDK

SEQ ID NO: 11 - protein, 8 aa, Mus musculus
TVRNVMDY

SEQ ID NO: 12 - DNA, 351 bp, Mus musculus
gaggttcagctccagcagtctgggactgtgctggcaaggcctggggcttcagtgaagatgtcctgcaaggcttctggctacacctttaccagctactggatgcactggataaaacagaggcctggacagggtctggaatggattggcgctatttatcctggaaatagtgatactaaatacaaccagaagttcaaggacaaggccaaactgactgcagtcacatctgccagcactgcctacatggagctcagcagcctgacaaatgaggactctgcggtctattactgtacatctacggtacggaatgttatggactactggggtcaaggaacctcagtcaccgtctcctca

SEQ ID NO: 13 - protein, 107 aa, Mus musculus
EIQMTQSPSSMSASLGDRITITCQATQDIVKSLNWYQQKPGKPPSFLIYYTAQLAEGVPSRFSGSGSGSDYSLTISNLESEDFADYYCLQFYEFPPTFGGGTKLEIK

SEQ ID NO: 14 - protein, 11 aa, Mus musculus
QATQDIVKSLN

SEQ ID NO: 15 - protein, 7 aa, Mus musculus
YTAQLAE

SEQ ID NO: 16 - protein, 9 aa, Mus musculus
LQFYEFPPT

SEQ ID NO: 17 - DNA, 321 bp, Mus musculus
gaaatccagatgacccagtctccatcctctatgtctgcatctctgggagacagaataaccatcacttgccaggcaactcaagacattgttaagagtttaaactggtatcaacaaaaaccagggaaacccccttcattcctgatctattatacagctcaactggcagaaggggtcccatcaaggttcagtggcagtgggtctgggtcagactattctctgacaatcagcaacctggagtctgaagattttgcagactattactgtctacagttttatgagtttcctccgacgttcggtggaggcaccaagctggaaatcaaa

SEQ ID NO: 18 - protein, 107 aa, Mus musculus [sequence omitted]

SEQ ID NO: 19 - protein, 107 aa, Artificial Sequence
  Synthetic
DIQMTQSPSSLSASVGDRVTITCQATQDIVKSLNWYQQKPGKPPKFLIYYTAQLAEGVPSRFSGSGSGTDYTLTISSLQSEDFATYYCLQFYEFPPTFGGGTKVEIK

SEQ ID NO: 20 - protein, 107 aa, Artificial Sequence
  Synthetic
DIQMTQSPSSLSASVGDRVTITCQATQDIVKSLNWYQQKPGKPPKFLIYYTAQLAEGVPSRFSGSGSGTDYTLTISSLQPEDFATYYCLQFYEFPPTFGGGTKVEIK

SEQ ID NO: 21 - protein, 107 aa, Artificial Sequence
  Synthetic
DIQMTQSPSSLSASVGDRVTITCQATQDIVKSLNWYQQKPGKAPKFLIYYTAQLAEGVPSRFSGSGSGTDYTLTISSLQPEDFATYYCLQFYEFPPTFGGGTKVEIK

SEQ ID NO: 22 - protein, 107 aa, Artificial Sequence
  Synthetic
DIQMTQSPSSLSASVGDRVTITCQATQDIVKSLNWYQQKPGKPPKFLIYYTAQLAEGVPSRFSGSGSGTDFTLTISSLQPEDFATYYCLQFYEFPPTFGGGTKVEIK

SEQ ID NO: 23 - protein, 107 aa, Artificial Sequence
  Synthetic
DIQMTQSPSSLSASVGDRVTITCQATQDIVKSLNWYQQKPGKPPKFAIYYTAQLAEGVPSRFSGSGSGTDYTLTISSLQPEDFATYYCLQFYEFPPTFGGGTKVEIK

SEQ ID NO: 24 - protein, 214 aa, Artificial Sequence
  Synthetic
DIQMTQSPSSLSASVGDRVTITCQATQDIVKSLNWYQQKPGKPPKFLIYYTAQLAEGVPSRFSGSGSGTDYTLTISSLQSEDFATYYCLQFYEFPPTFGGGTKVEIKRTVAAPSVFIFPPSDEQLKSGTASVVCLLNNFYPREAKVQWKVDNALQSGNSQESVTEQDSKDSTYSLSSTLTLSKADYEKHKVYACEVTHQGLSSPVTKSFNRGEC

SEQ ID NO: 25 - protein, 214 aa, Artificial Sequence
  Synthetic
DIQMTQSPSSLSASVGDRVTITCQATQDIVKSLNWYQQKPGKPPKFLIYYTAQLAEGVPSRFSGSGSGTDYTLTISSLQPEDFATYYCLQFYEFPPTFGGGTKVEIKRTVAAPSVFIFPPSDEQLKSGTASVVCLLNNFYPREAKVQWKVDNALQSGNSQESVTEQDSKDSTYSLSSTLTLSKADYEKHKVYACEVTHQGLSSPVTKSFNRGEC

SEQ ID NO: 26 - protein, 214 aa, Artificial Sequence
  Synthetic
DIQMTQSPSSLSASVGDRVTITCQATQDIVKSLNWYQQKPGKAPKFLIYYTAQLAEGVPSRFSGSGSGTDYTLTISSLQPEDFATYYCLQFYEFPPTFGGGTKVEIKRTVAAPSVFIFPPSDEQLKSGTASVVCLLNNFYPREAKVQWKVDNALQSGNSQESVTEQDSKDSTYSLSSTLTLSKADYEKHKVYACEVTHQGLSSPVTKSFNRGEC

SEQ ID NO: 27 - protein, 214 aa, Artificial Sequence
  Synthetic
DIQMTQSPSSLSASVGDRVTITCQATQDIVKSLNWYQQKPGKPPKFLIYYTAQLAEGVPSRFSGSGSGTDFTLTISSLQPEDFATYYCLQFYEFPPTFGGGTKVEIKRTVAAPSVFIFPPSDEQLKSGTASVVCLLNNFYPREAKVQWKVDNALQSGNSQESVTEQDSKDSTYSLSSTLTLSKADYEKHKVYACEVTHQGLSSPVTKSFNRGEC

SEQ ID NO: 28 - protein, 214 aa, Artificial Sequence; identical to SEQ ID NO: 27
  Synthetic

SEQ ID NO: 29 - protein, 117 aa, Mus musculus
EVQLQQSGTVLARPGASVKMSCKVSGYPFTSYWMHWVKQRPGQGLEWIGAIYPGKSDTEYNPNFKGKAKLTAVTSATTAYMELSSLTNEDSAVYYCTSTWTHYFDYWGQGTTLTVSS

SEQ ID NO: 30 - protein, 17 aa, Mus musculus
AIYPGKSDTEYNPNFKG

SEQ ID NO: 31 - DNA, 351 bp, Mus musculus
gaggttcagctccagcagtctgggactgttctggcaaggcctggggcttcagtgaagatgtcctgcaaggtttctggctacccctttaccagctactggatgcactgggtaaaacagaggcctggacagggtctggaatggattggcgctatttatcctggaaaaagtgacactgaatacaacccgaacttcaagggcaaggccaaactgactgcagtcacatctgccaccactgcctacatggagctcagcagcctgacaaatgaggactctgcggtctattactgtacaagtacctggacccactactttgactactggggccaaggcaccactctcacagtctcctca

SEQ ID NO: 32 - protein, 330 aa, Mus musculus [sequence omitted]

SEQ ID NO: 33 - protein, 330 aa, Mus musculus
ASTKGPSVFPLAPSSKSTSGGTAALGCLVKDYFPEPVTVSWNSGALTSGVHTFPAVLQSSGLYSLSSVVTVPSSSLGTQTYICNVNHKPSNTKVDKKVEPKSCDKTHTCPPCPAPELLGGPDVFLFPPKPKDTLMISRTPEVTCVVVDVSHEDPEVKFNWYVDGVEVHNAKTKPREEQYNSTYRVVSVLTVLHQDWLNGKEYKCKVSNKALPLPEEKTISKAKGQPREPQVYTLPPSRDELTKNQVSLTCLVKGFYPSDIAVEWESNGQPENNYKTTPPVLDSDGSFFLYSKLTVDKSRWQQGNVFSCSVMHEALHNHYTQKSLSLSPGK

SEQ ID NO: 34 - protein, 117 aa, Artificial Sequence
  Synthetic
EVQLVQSGAEVKKPGASVKVSCKVSGYPFTSYWMHWVRQAPGQGLEWIGAIYPGKSDTEYAPKFQGRVTLTADTSTSTAYMELSSLRSEDTAVYYCTSTWTHYFDYWGQGTTVTVSS

SEQ ID NO: 35 - protein, 117 aa, Artificial Sequence
  Synthetic
QVQLVQSGAEVKKPGASVKVSCKVSGYPFTSYWMHWVRQAPGQGLEWMGAIYPGKSDTEYAQKFQGRVTLTADTSTSTAYMELSSLRSEDTAVYYCTSTWTHYFDYWGQGTTVTVSS

SEQ ID NO: 36 - protein, 117 aa, Artificial Sequence
  Synthetic
QVQLVQSGAEVKKPGASVKVSCKVSGYPFTSYWMHWVRQAPGQGLEWMGAIYPGKSDTEYAQKFQGRVTLTADTSTSTAYMELSSLRSEDTATYYCTSTWTHYFDYWGQGTTVTVSS

SEQ ID NO: 37 - protein, 117 aa, Artificial Sequence
  Synthetic
QVQLVQSGAEVKKPGASVKVSCKVSGYPFTSYYMHWVRQAPGQGLEWMGAIYPGKSDTEYAQKFQGRVTLTADTSTSTAYMELSSLRSEDTATYYCTSTWTHYFDYWGQGTTVTVSS

SEQ ID NO: 38 - protein, 447 aa, Artificial Sequence
  Synthetic
EVQLVQSGAEVKKPGASVKVSCKVSGYPFTSYWMHWVRQAPGQGLEWIGAIYPGKSDTEYAPKFQGRVTLTADTSTSTAYMELSSLRSEDTAVYYCTSTWTHYFDYWGQGTTVTVSSASTKGPSVFPLAPSSKSTSGGTAALGCLVKDYFPEPVTVSWNSGALTSGVHTFPAVLQSSGLYSLSSVVTVPSSSLGTQTYICNVNHKPSNTKVDKKVEPKSCDKTHTCPPCPAPELLGGPSVFLFPPKPKDTLMISRTPEVTCVVVDVSHEDPEVKFNWYVDGVEVHNAKTKPREEQYNSTYRVVSVLTVLHQDWLNGKEYKCKVSNKALPAPIEKTISKAKGQPREPQVYTLPPSRDELTKNQVSLTCLVKGFYPSDIAVEWESNGQPENNYKTTPPVLDSDGSFFLYSKLTVDKSRWQQGNVFSCSVMHEALHNHYTQKSLSLSPGK

SEQ ID NO: 39 - protein, 447 aa, Artificial Sequence
  Synthetic
QVQLVQSGAEVKKPGASVKVSCKVSGYPFTSYWMHWVRQAPGQGLEWMGAIYPGKSDTEYAQKFQGRVTLTADTSTSTAYMELSSLRSEDTAVYYCTSTWTHYFDYWGQGTTVTVSSASTKGPSVFPLAPSSKSTSGGTAALGCLVKDYFPEPVTVSWNSGALTSGVHTFPAVLQSSGLYSLSSVVTVPSSSLGTQTYICNVNHKPSNTKVDKKVEPKSCDKTHTCPPCPAPELLGGPSVFLFPPKPKDTLMISRTPEVTCVVVDVSHEDPEVKFNWYVDGVEVHNAKTKPREEQYNSTYRVVSVLTVLHQDWLNGKEYKCKVSNKALPAPIEKTISKAKGQPREPQVYTLPPSRDELTKNQVSLTCLVKGFYPSDIAVEWESNGQPENNYKTTPPVLDSDGSFFLYSKLTVDKSRWQQGNVFSCSVMHEALHNHYTQKSLSLSPGK

SEQ ID NO: 40 - protein, 447 aa, Artificial Sequence
  Synthetic
QVQLVQSGAEVKKPGASVKVSCKVSGYPFTSYWMHWVRQAPGQGLEWMGAIYPGKSDTEYAQKFQGRVTLTADTSTSTAYMELSSLRSEDTATYYCTSTWTHYFDYWGQGTTVTVSSASTKGPSVFPLAPSSKSTSGGTAALGCLVKDYFPEPVTVSWNSGALTSGVHTFPAVLQSSGLYSLSSVVTVPSSSLGTQTYICNVNHKPSNTKVDKKVEPKSCDKTHTCPPCPAPELLGGPSVFLFPPKPKDTLMISRTPEVTCVVVDVSHEDPEVKFNWYVDGVEVHNAKTKPREEQYNSTYRVVSVLTVLHQDWLNGKEYKCKVSNKALPAPIEKTISKAKGQPREPQVYTLPPSRDELTKNQVSLTCLVKGFYPSDIAVEWESNGQPENNYKTTPPVLDSDGSFFLYSKLTVDKSRWQQGNVFSCSVMHEALHNHYTQKSLSLSPGK

SEQ ID NO: 41 - protein, 447 aa, Artificial Sequence
  Synthetic
QVQLVQSGAEVKKPGASVKVSCKVSGYPFTSYYMHWVRQAPGQGLEWMGAIYPGKSDTEYAQKFQGRVTLTADTSTSTAYMELSSLRSEDTATYYCTSTWTHYFDYWGQGTTVTVSSASTKGPSVFPLAPSSKSTSGGTAALGCLVKDYFPEPVTVSWNSGALTSGVHTFPAVLQSSGLYSLSSVVTVPSSSLGTQTYICNVNHKPSNTKVDKKVEPKSCDKTHTCPPCPAPELLGGPSVFLFPPKPKDTLMISRTPEVTCVVVDVSHEDPEVKFNWYVDGVEVHNAKTKPREEQYNSTYRVVSVLTVLHQDWLNGKEYKCKVSNKALPAPIEKTISKAKGQPREPQVYTLPPSRDELTKNQVSLTCLVKGFYPSDIAVEWESNGQPENNYKTTPPVLDSDGSFFLYSKLTVDKSRWQQGNVFSCSVMHEALHNHYTQKSLSLSPGK

SEQ ID NO: 42 - protein, 447 aa, Artificial Sequence
  Synthetic
EVQLVQSGAEVKKPGASVKVSCKVSGYPFTSYWMHWVRQAPGQGLEWIGAIYPGKSDTEYAPKFQGRVTLTADTSTSTAYMELSSLRSEDTAVYYCTSTWTHYFDYWGQGTTVTVSSASTKGPSVFPLAPSSKSTSGGTAALGCLVKDYFPEPVTVSWNSGALTSGVHTFPAVLQSSGLYSLSSVVTVPSSSLGTQTYICNVNHKPSNTKVDKKVEPKSCDKTHTCPPCPAPELLGGPDVFLFPPKPKDTLMISRTPEVTCVVVDVSHEDPEVKFNWYVDGVEVHNAKTKPREEQYNSTYRVVSVLTVLHQDWLNGKEYKCKVSNKALPLPEEKTISKAKGQPREPQVYTLPPSRDELTKNQVSLTCLVKGFYPSDIAVEWESNGQPENNYKTTPPVLDSDGSFFLYSKLTVDKSRWQQGNVFSCSVMHEALHNHYTQKSLSLSPGK

SEQ ID NO: 43 - protein, 447 aa, Artificial Sequence
  Synthetic
QVQLVQSGAEVKKPGASVKVSCKVSGYPFTSYWMHWVRQAPGQGLEWMGAIYPGKSDTEYAQKFQGRVTLTADTSTSTAYMELSSLRSEDTAVYYCTSTWTHYFDYWGQGTTVTVSSASTKGPSVFPLAPSSKSTSGGTAALGCLVKDYFPEPVTVSWNSGALTSGVHTFPAVLQSSGLYSLSSVVTVPSSSLGTQTYICNVNHKPSNTKVDKKVEPKSCDKTHTCPPCPAPELLGGPDVFLFPPKPKDTLMISRTPEVTCVVVDVSHEDPEVKFNWYVDGVEVHNAKTKPREEQYNSTYRVVSVLTVLHQDWLNGKEYKCKVSNKALPLPEEKTISKAKGQPREPQVYTLPPSRDELTKNQVSLTCLVKGFYPSDIAVEWESNGQPENNYKTTPPVLDSDGSFFLYSKLTVDKSRWQQGNVFSCSVMHEALHNHYTQKSLSLSPGK

SEQ ID NO: 44 - protein, 447 aa, Artificial Sequence
  Synthetic
QVQLVQSGAEVKKPGASVKVSCKVSGYPFTSYWMHWVRQAPGQGLEWMGAIYPGKSDTEYAQKFQGRVTLTADTSTSTAYMELSSLRSEDTATYYCTSTWTHYFDYWGQGTTVTVSSASTKGPSVFPLAPSSKSTSGGTAALGCLVKDYFPEPVTVSWNSGALTSGVHTFPAVLQSSGLYSLSSVVTVPSSSLGTQTYICNVNHKPSNTKVDKKVEPKSCDKTHTCPPCPAPELLGGPDVFLFPPKPKDTLMISRTPEVTCVVVDVSHEDPEVKFNWYVDGVEVHNAKTKPREEQYNSTYRVVSVLTVLHQDWLNGKEYKCKVSNKALPLPEEKTISKAKGQPREPQVYTLPPSRDELTKNQVSLTCLVKGFYPSDIAVEWESNGQPENNYKTTPPVLDSDGSFFLYSKLTVDKSRWQQGNVFSCSVMHEALHNHYTQKSLSLSPGK

SEQ ID NO: 45 - protein, 447 aa, Artificial Sequence
  Synthetic
QVQLVQSGAEVKKPGASVKVSCKVSGYPFTSYYMHWVRQAPGQGLEWMGAIYPGKSDTEYAQKFQGRVTLTADTSTSTAYMELSSLRSEDTATYYCTSTWTHYFDYWGQGTTVTVSSASTKGPSVFPLAPSSKSTSGGTAALGCLVKDYFPEPVTVSWNSGALTSGVHTFPAVLQSSGLYSLSSVVTVPSSSLGTQTYICNVNHKPSNTKVDKKVEPKSCDKTHTCPPCPAPELLGGPDVFLFPPKPKDTLMISRTPEVTCVVVDVSHEDPEVKFNWYVDGVEVHNAKTKPREEQYNSTYRVVSVLTVLHQDWLNGKEYKCKVSNKALPLPEEKTISKAKGQPREPQVYTLPPSRDELTKNQVSLTCLVKGFYPSDIAVEWESNGQPENNYKTTPPVLDSDGSFFLYSKLTVDKSRWQQGNVFSCSVMHEALHNHYTQKSLSLSPGK

SEQ ID NO: 46 - protein, 107 aa, Mus musculus
EIQMTQSPSSMSASLGDTITITCQATQDIVKSLNWYQQKPGKPPSFLIYYTTQLAEGVPSRFSGSGSGSDYSLTISNLDSEDFADYYCLQFYEFPPTFGGGTKLEIK

SEQ ID NO: 47 - protein, 8 aa, Mus musculus
YYTTQLAE

SEQ ID NO: 48 - DNA, 321 bp, Mus musculus
gaaatccagatgacccagtctccatcctctatgtctgcatctctgggagacacaataaccatcacttgccaggcaactcaagacattgttaagagtttaaactggtatcaacaaaaaccagggaaacccccttcattcctgatctattatacaactcaactggcagaaggggtcccatcaaggttcagtggcagtgggtctgggtcagactattctctgacaatcagcaacctggactctgaagattttgcagactattactgtctacagttttatgagtttcctccgacgttcggtggaggcaccaagctggaaatcaaa

SEQ ID NO: 49 - protein, 117 aa, Mus musculus
EVQLQQSGTVLARPGASVKMSCKASGYTFSSYWMHWVKQRPGQGLEWIGAIYPGKSDTSYNQKFQGKAKLTAVTSASTAFMELTSLTNEDSAVYYCTSTWTHYFDYWGQGTTLTVSS

SEQ ID NO: 50 - protein, 17 aa, Mus musculus
AIYPGKSDTEYNPNFKG

SEQ ID NO: 51 - DNA, 351 bp, Mus musculus
gaggttcagctccagcagtctgggactgttctggcaaggcctggggcttcagtgaagatgtcctgcaaggcttctggctacaccttttccagctactggatgcactgggtaaaacagaggcctggacagggtctggaatggattggcgctatttatcctggaaaaagtgatactagctacaaccagaagttccagggcaaggccaaactgactgcagtcacatctgccagcactgccttcatggagctcaccagcctgacaaatgaggactctgcggtctattactgtacaagtacctggacccactactttgactactggggccaaggcaccactctcacagtctcctca

SEQ ID NO: 52 - protein, 107 aa, Mus musculus
DIQMTQTTSSLSASLGDRVTISCRASQDISNYLNWYQQKPDGTIKLLIYYTSRLHSGVPSRFSGSGSGSDYSLTISNLEQEDIATYFCQQGNTLPWTFGGGTKLEFK

SEQ ID NO: 53 - protein, 11 aa, Mus musculus
RASQDISNYLN

SEQ ID NO: 54 - protein, 7 aa, Mus musculus
YTSRLHS

SEQ ID NO: 55 - protein, 9 aa, Mus musculus
QQGNTLPWT

SEQ ID NO: 56 - DNA, 321 bp, Mus musculus
gatatccagatgacacaaactacatcctccctgtctgcctctctgggagacagagtcaccatcagttgcagggcaagtcaggacattagcaattatttaaactggtatcagcagaaaccagatggaactattaaactcctgatctattacacatcaagattacattcaggagtcccatcaaggttcagtggcagtgggtctggatcagattattctctcaccattagcaacctggagcaagaagatattgccacttacttttgccaacagggtaatacgcttccgtggacgttcggtggaggcaccaagctggaattcaaa

SEQ ID NO: 57 - protein, 214 aa, Mus musculus
DIQMTQSPSSLSASVGDRVTITCRASQDISNYLNWYQQKPGKTIKLLIYYTSRLHSGVPSRFSGSGSGTDYTLTISSLQPEDFATYFCQQGNTLPWTFGQGTKLEIKRTVAAPSVFIFPPSDEQLKSGTASVVCLLNNFYPREAKVQWKVDNALQSGNSQESVTEQDSKDSTYSLSSTLTLSKADYEKHKVYACEVTHQGLSSPVTKSFNRGEC

SEQ ID NO: 58 - protein, 107 aa, Artificial Sequence
  Synthetic
DIQMTQSPSSLSASVGDRVTITCRASQDISNYLNWYQQKPGKTIKLLIYYTSRLHSGVPSRFSGSGSGTDYTLTISSLQPEDFATYFCQQGNTLPWTFGQGTKLEIK

SEQ ID NO: 59 - protein, 107 aa, Artificial Sequence
  Synthetic
DIQMTQSPSSLSASVGDRVTITCRASQDISNYLNWYQQKPGKAPKLLIYYTSRLHSGVPSRFSGSGSGTDYTLTISSLQPEDFATYFCQQGNTLPWTFGQGTKLEIK

SEQ ID NO: 60 - protein, 107 aa, Artificial Sequence
  Synthetic
DIQMTQSPSSLSASVGDRVTITCRASQDISNYLNWYQQKPGKAPKLLIYYTSRLHSGVPSRFSGSGSGTDYTLTISSLQPEDFATYFCQQGQTLPWTFGQGTKLEIK

SEQ ID NO: 61 - protein, 107 aa, Artificial Sequence
  Synthetic
DIQMTQSPSSLSASVGDRVTITCRASQDISNYLNWYQQKPGKAPKLLIYYTSRLHSGVPSRFSGSGSGTDYTLTISSLQPEDFATYFCQQGSTLPWTFGQGTKLEIK

SEQ ID NO: 62 - protein, 214 aa, Artificial Sequence
  Synthetic
DIQMTQSPSSLSASVGDRVTITCRASQDISNYLNWYQQKPGKAPKLLIYYTSRLHSGVPSRFSGSGSGTDYTLTISSLQPEDFATYFCQQGNTLPWTFGQGTKLEIKRTVAAPSVFIFPPSDEQLKSGTASVVCLLNNFYPREAKVQWKVDNALQSGNSQESVTEQDSKDSTYSLSSTLTLSKADYEKHKVYACEVTHQGLSSPVTKSFNRGEC

SEQ ID NO: 63 - protein, 214 aa, Artificial Sequence
  Synthetic
DIQMTQSPSSLSASVGDRVTITCRASQDISNYLNWYQQKPGKAPKLLIYYTSRLHSGVPSRFSGSGSGTDYTLTISSLQPEDFATYFCQQGQTLPWTFGQGTKLEIKRTVAAPSVFIFPPSDEQLKSGTASVVCLLNNFYPREAKVQWKVDNALQSGNSQESVTEQDSKDSTYSLSSTLTLSKADYEKHKVYACEVTHQGLSSPVTKSFNRGEC

SEQ ID NO: 64 - protein, 214 aa, Artificial Sequence
  Synthetic
DIQMTQSPSSLSASVGDRVTITCRASQDISNYLNWYQQKPGKAPKLLIYYTSRLHSGVPSRFSGSGSGTDYTLTISSLQPEDFATYFCQQGSTLPWTFGQGTKLEIKRTVAAPSVFIFPPSDEQLKSGTASVVCLLNNFYPREAKVQWKVDNALQSGNSQESVTEQDSKDSTYSLSSTLTLSKADYEKHKVYACEVTHQGLSSPVTKSFNRGEC

SEQ ID NO: 65 - protein, 116 aa, Mus musculus
EVQLQQSGPELVKPGASVKMSCKASGYTFTDYYMNWVRQSHGKSLEWIGRVNPSNGGTNYNQKFKGKATLTVDKSLSTAYMQLSSLTSEDSAVYYCARRHNYADFWGQGTTLTVSS

SEQ ID NO: 66 - protein, 5 aa, Mus musculus
DYYMN

SEQ ID NO: 67 - protein, 17 aa, Mus musculus
RVNPSNGGTNYNQKFKG

SEQ ID NO: 68 - protein, 7 aa, Mus musculus
RHNYADF

SEQ ID NO: 69 - DNA, 348 bp, Mus musculus
gaggtccagctgcaacagtctggacctgagctggtgaagcctggggcttcagtgaagatgtcctgtaaggcttctggatacacattcactgactactacatgaactgggtgaggcagagtcatggaaagagccttgagtggattggacgtgttaatcctagcaatggtggtactaactacaaccagaaattcaagggcaaggccacattgacagtagacaaatccctcagcacagcctacatgcagctcagcagcctgacatctgaggactctgcggtctattactgtgcaagacgacataactacgcagacttctggggccaaggcaccactctcacagtctcctca

SEQ ID NO: 70 - protein, 116 aa, Artificial Sequence
  Synthetic
EVQLVQSGAEVKKPGASVKVSCKASGYTFTDYYMNWVRQAPGQGLEWIGRVNPSNGGTNYAQKFQGRVTLTVDKSTSTAYMELSSLRSEDTAVYYCARRHNYADFWGQGTTVTVSS

SEQ ID NO: 71 - protein, 116 aa, Artificial Sequence
  Synthetic
QVQLVQSGAEVKKPGASVKVSCKASGYTFTDYYMNWVRQAPGQGLEWMGRVNPANGGTNYAQKFQGRVTLTVDTSTSTAYMELSSLRSEDTAVYYCARRHNYADFWGQGTTVTVSS

SEQ ID NO: 72 - protein, 116 aa, Artificial Sequence
  Synthetic
QVQLVQSGAEVKKPGASVKVSCKASGYTFTDYYMNWVRQAPGQGLEWMGRVNPSSGGTNYAQKFQGRVTLTVDTSTSTAYMELSSLRSEDTAVYYCARRHNYADFWGQGTTVTVSS

SEQ ID NO: 73 - protein, 116 aa, Artificial Sequence
  Synthetic
QVQLVQSGAEVKKPGASVKVSCKASGYTFTDYYMNWVRQAPGQGLEWMGRVNPSNGGTNYAQKFQGRVTLTVDTSKSTAYMELSSLRSEDTAVYYCARRHNYADFWGQGTTVTVSS

SEQ ID NO: 74 - protein, 116 aa, Artificial Sequence
  Synthetic
QVQLVQSGAEVKKPGASVKVSCKASGYTFTDYYMNWVRQAPGQGLEWMGRVNPSSGGTNYAQKFQGRVTLTVDTSKSTAYMELSSLRSEDTAVYYCARRHNYADFWGQGTTVTVSS

SEQ ID NO: 75 - protein, 446 aa, Artificial Sequence
  Synthetic
EVQLVQSGAEVKKPGASVKVSCKASGYTFTDYYMNWVRQAPGQGLEWIGRVNPSNGGTNYAQKFQGRVTLTVDKSTSTAYMELSSLRSEDTAVYYCARRHNYADFWGQGTTVTVSSASTKGPSVFPLAPSSKSTSGGTAALGCLVKDYFPEPVTVSWNSGALTSGVHTFPAVLQSSGLYSLSSVVTVPSSSLGTQTYICNVNHKPSNTKVDKKVEPKSCDKTHTCPPCPAPELLGGPSVFLFPPKPKDTLMISRTPEVTCVVVDVSHEDPEVKFNWYVDGVEVHNAKTKPREEQYNSTYRVVSVLTVLHQDWLNGKEYKCKVSNKALPAPIEKTISKAKGQPREPQVYTLPPSRDELTKNQVSLTCLVKGFYPSDIAVEWESNGQPENNYKTTPPVLDSDGSFFLYSKLTVDKSRWQQGNVFSCSVMHEALHNHYTQKSLSLSPGK

SEQ ID NO: 76 - protein, 446 aa, Artificial Sequence
  Synthetic
QVQLVQSGAEVKKPGASVKVSCKASGYTFTDYYMNWVRQAPGQGLEWMGRVNPANGGTNYAQKFQGRVTLTVDTSTSTAYMELSSLRSEDTAVYYCARRHNYADFWGQGTTVTVSSASTKGPSVFPLAPSSKSTSGGTAALGCLVKDYFPEPVTVSWNSGALTSGVHTFPAVLQSSGLYSLSSVVTVPSSSLGTQTYICNVNHKPSNTKVDKKVEPKSCDKTHTCPPCPAPELLGGPSVFLFPPKPKDTLMISRTPEVTCVVVDVSHEDPEVKFNWYVDGVEVHNAKTKPREEQYNSTYRVVSVLTVLHQDWLNGKEYKCKVSNKALPAPIEKTISKAKGQPREPQVYTLPPSRDELTKNQVSLTCLVKGFYPSDIAVEWESNGQPENNYKTTPPVLDSDGSFFLYSKLTVDKSRWQQGNVFSCSVMHEALHNHYTQKSLSLSPGK

SEQ ID NO: 77 - protein, 446 aa, Artificial Sequence
  Synthetic
QVQLVQSGAEVKKPGASVKVSCKASGYTFTDYYMNWVRQAPGQGLEWMGRVNPSSGGTNYAQKFQGRVTLTVDTSTSTAYMELSSLRSEDTAVYYCARRHNYADFWGQGTTVTVSSASTKGPSVFPLAPSSKSTSGGTAALGCLVKDYFPEPVTVSWNSGALTSGVHTFPAVLQSSGLYSLSSVVTVPSSSLGTQTYICNVNHKPSNTKVDKKVEPKSCDKTHTCPPCPAPELLGGPSVFLFPPKPKDTLMISRTPEVTCVVVDVSHEDPEVKFNWYVDGVEVHNAKTKPREEQYNSTYRVVSVLTVLHQDWLNGKEYKCKVSNKALPAPIEKTISKAKGQPREPQVYTLPPSRDELTKNQVSLTCLVKGFYPSDIAVEWESNGQPENNYKTTPPVLDSDGSFFLYSKLTVDKSRWQQGNVFSCSVMHEALHNHYTQKSLSLSPGK

SEQ ID NO: 78 - protein, 446 aa, Artificial Sequence
  Synthetic
QVQLVQSGAEVKKPGASVKVSCKASGYTFTDYYMNWVRQAPGQGLEWMGRVNPSNGGTNYAQKFQGRVTLTVDTSKSTAYMELSSLRSEDTAVYYCARRHNYADFWGQGTTVTVSSASTKGPSVFPLAPSSKSTSGGTAALGCLVKDYFPEPVTVSWNSGALTSGVHTFPAVLQSSGLYSLSSVVTVPSSSLGTQTYICNVNHKPSNTKVDKKVEPKSCDKTHTCPPCPAPELLGGPSVFLFPPKPKDTLMISRTPEVTCVVVDVSHEDPEVKFNWYVDGVEVHNAKTKPREEQYNSTYRVVSVLTVLHQDWLNGKEYKCKVSNKALPAPIEKTISKAKGQPREPQVYTLPPSRDELTKNQVSLTCLVKGFYPSDIAVEWESNGQPENNYKTTPPVLDSDGSFFLYSKLTVDKSRWQQGNVFSCSVMHEALHNHYTQKSLSLSPGK

SEQ ID NO: 79 - protein, 446 aa, Artificial Sequence
  Synthetic
QVQLVQSGAEVKKPGASVKVSCKASGYTFTDYYMNWVRQAPGQGLEWMGRVNPSSGGTNYAQKFQGRVTLTVDTSKSTAYMELSSLRSEDTAVYYCARRHNYADFWGQGTTVTVSSASTKGPSVFPLAPSSKSTSGGTAALGCLVKDYFPEPVTVSWNSGALTSGVHTFPAVLQSSGLYSLSSVVTVPSSSLGTQTYICNVNHKPSNTKVDKKVEPKSCDKTHTCPPCPAPELLGGPSVFLFPPKPKDTLMISRTPEVTCVVVDVSHEDPEVKFNWYVDGVEVHNAKTKPREEQYNSTYRVVSVLTVLHQDWLNGKEYKCKVSNKALPAPIEKTISKAKGQPREPQVYTLPPSRDELTKNQVSLTCLVKGFYPSDIAVEWESNGQPENNYKTTPPVLDSDGSFFLYSKLTVDKSRWQQGNVFSCSVMHEALHNHYTQKSLSLSPGK

SEQ ID NO: 80 - protein, 446 aa, Artificial Sequence
  Synthetic
EVQLVQSGAEVKKPGASVKVSCKASGYTFTDYYMNWVRQAPGQGLEWIGRVNPSNGGTNYAQKFQGRVTLTVDKSTSTAYMELSSLRSEDTAVYYCARRHNYADFWGQGTTVTVSSASTKGPSVFPLAPSSKSTSGGTAALGCLVKDYFPEPVTVSWNSGALTSGVHTFPAVLQSSGLYSLSSVVTVPSSSLGTQTYICNVNHKPSNTKVDKKVEPKSCDKTHTCPPCPAPELLGGPDVFLFPPKPKDTLMISRTPEVTCVVVDVSHEDPEVKFNWYVDGVEVHNAKTKPREEQYNSTYRVVSVLTVLHQDWLNGKEYKCKVSNKALPLPEEKTISKAKGQPREPQVYTLPPSRDELTKNQVSLTCLVKGFYPSDIAVEWESNGQPENNYKTTPPVLDSDGSFFLYSKLTVDKSRWQQGNVFSCSVMHEALHNHYTQKSLSLSPGK

SEQ ID NO: 81 - protein, 446 aa, Artificial Sequence
  Synthetic
QVQLVQSGAEVKKPGASVKVSCKASGYTFTDYYMNWVRQAPGQGLEWMGRVNPANGGTNYAQKFQGRVTLTVDTSTSTAYMELSSLRSEDTAVYYCARRHNYADFWGQGTTVTVSSASTKGPSVFPLAPSSKSTSGGTAALGCLVKDYFPEPVTVSWNSGALTSGVHTFPAVLQSSGLYSLSSVVTVPSSSLGTQTYICNVNHKPSNTKVDKKVEPKSCDKTHTCPPCPAPELLGGPDVFLFPPKPKDTLMISRTPEVTCVVVDVSHEDPEVKFNWYVDGVEVHNAKTKPREEQYNSTYRVVSVLTVLHQDWLNGKEYKCKVSNKALPLPEEKTISKAKGQPREPQVYTLPPSRDELTKNQVSLTCLVKGFYPSDIAVEWESNGQPENNYKTTPPVLDSDGSFFLYSKLTVDKSRWQQGNVFSCSVMHEALHNHYTQKSLSLSPGK

SEQ ID NO: 82 - protein, 446 aa, Artificial Sequence
  Synthetic
QVQLVQSGAEVKKPGASVKVSCKASGYTFTDYYMNWVRQAPGQGLEWMGRVNPSSGGTNYAQKFQGRVTLTVDTSTSTAYMELSSLRSEDTAVYYCARRHNYADFWGQGTTVTVSSASTKGPSVFPLAPSSKSTSGGTAALGCLVKDYFPEPVTVSWNSGALTSGVHTFPAVLQSSGLYSLSSVVTVPSSSLGTQTYICNVNHKPSNTKVDKKVEPKSCDKTHTCPPCPAPELLGGPDVFLFPPKPKDTLMISRTPEVTCVVVDVSHEDPEVKFNWYVDGVEVHNAKTKPREEQYNSTYRVVSVLTVLHQDWLNGKEYKCKVSNKALPLPEEKTISKAKGQPREPQVYTLPPSRDELTKNQVSLTCLVKGFYPSDIAVEWESNGQPENNYKTTPPVLDSDGSFFLYSKLTVDKSRWQQGNVFSCSVMHEALHNHYTQKSLSLSPGK

SEQ ID NO: 83 - protein, 446 aa, Artificial Sequence
  Synthetic
QVQLVQSGAEVKKPGASVKVSCKASGYTFTDYYMNWVRQAPGQGLEWMGRVNPSNGGTNYAQKFQGRVTLTVDTSKSTAYMELSSLRSEDTAVYYCARRHNYADFWGQGTTVTVSSASTKGPSVFPLAPSSKSTSGGTAALGCLVKDYFPEPVTVSWNSGALTSGVHTFPAVLQSSGLYSLSSVVTVPSSSLGTQTYICNVNHKPSNTKVDKKVEPKSCDKTHTCPPCPAPELLGGPDVFLFPPKPKDTLMISRTPEVTCVVVDVSHEDPEVKFNWYVDGVEVHNAKTKPREEQYNSTYRVVSVLTVLHQDWLNGKEYKCKVSNKALPLPEEKTISKAKGQPREPQVYTLPPSRDELTKNQVSLTCLVKGFYPSDIAVEWESNGQPENNYKTTPPVLDSDGSFFLYSKLTVDKSRWQQGNVFSCSVMHEALHNHYTQKSLSLSPGK

SEQ ID NO: 84 - protein, 446 aa, Artificial Sequence
  Synthetic
QVQLVQSGAEVKKPGASVKVSCKASGYTFTDYYMNWVRQAPGQGLEWMGRVNPSSGGTNYAQKFQGRVTLTVDTSKSTAYMELSSLRSEDTAVYYCARRHNYADFWGQGTTVTVSSASTKGPSVFPLAPSSKSTSGGTAALGCLVKDYFPEPVTVSWNSGALTSGVHTFPAVLQSSGLYSLSSVVTVPSSSLGTQTYICNVNHKPSNTKVDKKVEPKSCDKTHTCPPCPAPELLGGPDVFLFPPKPKDTLMISRTPEVTCVVVDVSHEDPEVKFNWYVDGVEVHNAKTKPREEQYNSTYRVVSVLTVLHQDWLNGKEYKCKVSNKALPLPEEKTISKAKGQPREPQVYTLPPSRDELTKNQVSLTCLVKGFYPSDIAVEWESNGQPENNYKTTPPVLDSDGSFFLYSKLTVDKSRWQQGNVFSCSVMHEALHNHYTQKSLSLSPGK

SEQ ID NO: 85 - protein, 107 aa, Mus musculus
ETVMTQSHKIMSTSVGDRVTITCKASQDVRTAVAWYQQKPGQSPKLLISSASYQYTGVPDRFTGSGSGTDFTFTISSLQAEDLAVYYCHQYYNTPLTFGAGTKLELR

SEQ ID NO: 86 - protein, 7 aa, Mus musculus
SASYQYT

SEQ ID NO: 87 - protein, 9 aa, Mus musculus
HQYYNTPLT

SEQ ID NO: 88 - DNA, 321 bp, Mus musculus
gaaactgtgatgacccagtctcacaaaatcatgtccacttcagtaggagacagggtcaccatcacctgcaaggccagtcaggatgtgagaactgctgtggcctggtatcaacagaaaccaggacaatctcctaaattactaatttcctcggcatcctaccaatacactggagtccctgatcgcttcactggcagtggatctgggacggatttcactttcaccatcagcagtttgcaggctgaagacctggcagtttattactgtcatcagtattataatactccgctcacgttcggtgctgggaccaagctggagctgaga

SEQ ID NO: 89 - protein, 117 aa, Mus musculus
EVQLQQSGTVLARPGASVKMSCKASGYTFTSYWMHWVKQRPGQGLEWIGAIYPGKSDTTYNQKFEGKAKLTAVTSDSTAYMDLSSLTNEDSAVYYCTSSVRNAMDYWGQGTSVTVSS

SEQ ID NO: 90 - protein, 17 aa, Mus musculus
AIYPGKSDTTYNQKFEG

SEQ ID NO: 91 - protein, 8 aa, Mus musculus
SVRNAMDY

SEQ ID NO: 92 - DNA, 351 bp, Mus musculus
gaggttcagctccagcagtctgggactgtgctggcaaggcctggggcttcagtgaagatgtcctgcaaggcttctggctacaccttcaccagctactggatgcactgggtaaaacagaggcctggacagggtctggaatggattggcgctatttatcctggaaaaagtgatactacctacaaccagaagttcgagggcaaggccaaactgactgcagtcacatctgacagcacagcctacatggatctcagtagcctgacaaatgaggactctgcggtctattactgtacatcttcggttcggaatgctatggactactggggtcaaggaacctcagtcaccgtctcctca

SEQ ID NO: 93 - protein, 112 aa, Mus musculus
DVLMTQTPLSLPVSLGGQASISCRSSQIIVHSNGNTYLEWYLQKPGQSPKLLIYKVSNRFSGVPDRFSGSGSGTDFTLKISRVEAEDLGVYYCFQGSHVPWTFGGGTKLEIK

SEQ ID NO: 94 - protein, 16 aa, Mus musculus
RSSQIIVHSNGNTYLE

SEQ ID NO: 95 - protein, 7 aa, Mus musculus
KVSNRFS

SEQ ID NO: 96 - protein, 9 aa, Mus musculus
FQGSHVPWT

SEQ ID NO: 97 - DNA, 336 bp, Mus musculus
gatgttttgatgacccaaactccactctccctgcctgtcagtcttggaggtcaagcctccatctcttgcagatctagtcagatcattgtacatagtaatggaaacacctatttagaatggtacctgcagaaaccaggccagtctccaaagctcctgatctacaaagtttccaaccgattttctggggtcccagacaggttcagtggcagtggatcagggacagatttcacactcaagatcagcagagtggaggctgaggatctgggagtttattactgctttcaaggttcacatgttccgtggacgttcggtggaggcaccaagctggaaatcaaa

SEQ ID NO: 98 - protein, 119 aa, Mus musculus
QVQLQQPGAELVKPGASVKLSCKASGYTFISYWMHWVKQRPGQGLEWIGEIDPSDSYTYYNQKFKGKATLTVDKSSSTAYMQLSSLTSEDSAVYYCARRKTWDWYFDVWGAGTTVTVSS

SEQ ID NO: 99 - protein, 17 aa, Mus musculus
EIDPSDSYTYYNQKFKG

SEQ ID NO: 100 - protein, 10 aa, Mus musculus
RKTWDWYFDV

SEQ ID NO: 101 - DNA, 357 bp, Mus musculus
caggtccagctgcagcagcctggggctgaactggtgaagcctggggcttcagtgaagctgtcctgcaaggcttctggatacaccttcattagctactggatgcactgggtgaagcagaggcctggacaaggccttgagtggatcggagagattgatccttctgatagttatacttactacaatcaaaagttcaagggcaaggccacattgactgtagacaaatcctccagcacagcctacatgcaactcagcagcctgacatctgaggactctgcggtctattactgtgcaagaaggaaaacctgggactggtacttcgatgtctggggcgcagggaccacggtcaccgtctcctca

SEQ ID NO: 102 - protein, 106 aa, Mus musculus
DIVMTQSHKFMSTSVGDRVTITCKASQDVSTAVAWYQQKPGQSPKLLISSASYRYTGVPDRFTGSGSGTDFTFTISSVQAEDLAVYYCQQHYSTPTFGGGTKLEIR

SEQ ID NO: 103 - protein, 11 aa, Mus musculus
KASQDVSTAVA

SEQ ID NO: 104 - protein, 7 aa, Mus musculus
SASYRYT

SEQ ID NO: 105 - protein, 8 aa, Mus musculus
QQHYSTPT

SEQ ID NO: 106 - DNA, 318 bp, Mus musculus
gacattgtgatgacccagtctcacaaattcatgtccacatcagtaggagacagggtcactatcacctgcaaggccagtcaggatgtgagtactgctgtagcctggtatcaacagaaaccaggacagtctcctaaactactgatttcctcggcatcctaccggtacactggagtccctgatcgcttcactggcagtggatctgggacggatttcactttcaccatcagcagtgtgcaggctgaagacctggcagtttattactgtcagcaacattatagtactccgacgttcggtggaggcaccaagctggaaatcaga

SEQ ID NO: 107 - protein, 116 aa, Mus musculus
VQLQQSGTVLARPGASVKMSCKASGYTFTSYWMHWVKERPGQGLEWIGAIYPGDSDTRYNQKFKGRAKLTAVTSANTAYMELSSLTNDDSAVFYCTCTTAGVLDYWGQGTSVTVSS

SEQ ID NO: 108 - protein, 17 aa, Mus musculus
AIYPGDSDTRYNQKFKG

SEQ ID NO: 109 - protein, 8 aa, Mus musculus
TTAGVLDY

SEQ ID NO: 110 - DNA, 351 bp, Mus musculus
gaggttcagctccagcagtctgggactgtgctggcaaggcctggggcttcagtgaagatgtcctgcaaggcttctggctacacctttaccagctactggatgcactgggtaaaagagaggcctggacagggtctggaatggattggcgctatttatcctggagatagtgatactaggtataatcagaagttcaagggcagggccaaactgactgcagtcacatctgccaacactgcctacatggagctcagcagcctgacaaatgatgactctgcggtcttctactgtacatgtactacggctggtgttttggactactggggtcaaggaacctcagtcaccgtctcctca

SEQ ID NO: 111 - protein, 112 aa, Mus musculus
DVVMTQTPLSLPVSLGDQASISCTSSQSIVHGNGNTYLEWYLQKPGQSPKLLIYKVSNRFSGVPDRFSGSGSGTDFTLKISRVEAEDLGVYYCFQGSHVPYTFGGGTKLEIK

SEQ ID NO: 112 - protein, 16 aa, Mus musculus
TSSQSIVHGNGNTYLE

SEQ ID NO: 113 - protein, 9 aa, Mus musculus
FQGSHVPYT

SEQ ID NO: 114 - DNA, 336 bp, Mus musculus
gatgttgtgatgacccaaactccactctccctgcctgtcagtcttggagatcaggcctccatctcttgcacatctagtcagagcattgtacatggtaatggaaacacctatttagaatggtacctgcagaagccaggccagtctccaaagctcctgatctacaaagtttccaaccgattttctggggtcccagacaggttcagtggcagtggatcagggacagatttcacactcaagatcagcagagtggaggctgaggatctgggagtttattactgctttcaaggttcacatgttccgtacacgttcggaggggggaccaagctggaaataaaa

SEQ ID NO: 115 - protein, 123 aa, Mus musculus
QVQLQQPGAELVKPGASVKLSCKASGYSFTSYWMNWVKQRPGRGLEWIGRIHPSDSETHYNQKFKSKATLTVDKSSSTAYIQLSSLTSEDSAVYFCARYGLFYGNDGYAMDHWGQGTSVTVSS

SEQ ID NO: 116 - protein, 5 aa, Mus musculus
SYWMN

SEQ ID NO: 117 - protein, 17 aa, Mus musculus
RIHPSDSETHYNQKFKS

SEQ ID NO: 118 - protein, 14 aa, Mus musculus
YGLFYGNDGYAMDH

SEQ ID NO: 119 - DNA, 355 bp, Mus musculus
caggtccaactgcagcagcctggggctgaactggtgaagcctggggcttcagtgaagctgtcctgcaaggcttctggctactctttcaccagctactggatgaactgggtgaagcagaggcctggacgaggcctcgagtggattggaaggattcatccttctgatagtgaaactcactacaatcaaaagttcaagagcaaggccacactgactgtagacaaatcctccagcacagcctacatccaactcagcagcctgacatctgaggactctgcggtctatttttgtgcaagatacgggctcttctatggtaacgacggatatgctatggaccactggggtcaaggaacctcag

SEQ ID NO: 120 - protein, 107 aa, Mus musculus
DIQMTQTTSSLSASLGDRVTISCRASQDISFYLNWYQQKPDGTVKLLIYYTSRLHSGVPSRFSGSGSGTDYSLTISNLEQEDIATYFCQQGNTLPWTFGGGTKLEIK

SEQ ID NO: 121 - protein, 11 aa, Mus musculus
RASQDISFYLN

SEQ ID NO: 122 - DNA, 321 bp, Mus musculus
gatatccagatgacacagactacatcctccctgtctgcctctctgggagacagagtcaccatcagttgcagggcaagtcaggacattagcttttatttaaactggtatcagcagaaaccagatggaactgttaaactcctgatctactacacatcaagattacactcaggagtcccatcaaggttcagtggcagtgggtctggaacagattattctctcaccattagcaacctggagcaagaagatattgccacttacttttgccaacagggtaatacacttccgtggacgttcggtggaggcaccaagctggaaatcaaa

SEQ ID NO: 123 - protein, 116 aa, Mus musculus
EVQLQQSGPELVKPGASVKMSCKASGYTFTDYYMNWVKQSHGKSLEWIGRVNPSNGGTSYNQKFKGKATLTVDKSLSAAYMQLNSLTSEDSAVYYCARRHNYPDYWGQGTTLTVSS

SEQ ID NO: 124 - protein, 17 aa, Mus musculus
RVNPSNGGTSYNQKFKG

SEQ ID NO: 125 - protein, 7 aa, Mus musculus
RHNYPDY

SEQ ID NO: 126 - DNA, 348 bp, Mus musculus
gaggtccagctgcaacagtctggacctgaactggtgaagcctggggcttcagtgaagatgtcctgtaaggcttctggatacacattcactgactactacatgaactgggtgaagcagagtcatggaaagagccttgagtggattggacgtgttaatcctagcaatggtggtactagctacaaccagaagttcaagggcaaggccacattgacagtagacaaatccctcagcgcagcctatatgcagctcaacagcctgacatctgaggactctgcggtctattactgtgcaagaaggcataactaccctgactactggggccaaggcaccactctcacagtctcctca

SEQ ID NO: 127 - DNA, 320 bp, Mus musculus
gaaatccagatgacccagtctccatcctctatgtctgcatctctgggagacagaataaccatcacttgccaggcaactcaagacattgttaagagtttaaactggtatcaacaaaaaccagggaaacccccttcattcctgatctattatacagctcaactggcagaaggggtcccgtcaaggttcagtggcagtgggtctgggtcagactattctctgacaatcagcaacctggagtctgaagattttgcagactattactgtctacagttttatgagtttcctccgacgttcggtggaggcaccaagctggaaatcaa

SEQ ID NO: 128 - protein, 117 aa, Mus musculus
EVQLQQSGTVLARPGASVKMSCKASGYPFTSYWMHWVKQRPGQGLEWIGAIYPGNSDTRYNPNFKGKANLTAVTSATTAYMELSSLTNEESAVYYCTSTWTHYFDYWGQGTTLTVSS

SEQ ID NO: 129 - protein, 17 aa, Mus musculus
AIYPGNSDTRYNPNFKG

SEQ ID NO: 130 - protein, 8 aa, Mus musculus
TWTHYFDY

SEQ ID NO: 131 - DNA, 351 bp, Mus musculus
gaggttcagctccagcagtctgggactgtgctggcaaggcctggggcttcagtgaagatgtcctgcaaggcttctggctacccctttaccagctactggatgcactgggtaaagcagaggcctggacagggtctggaatggattggcgctatttatcctggaaatagtgatactaggtacaacccgaatttcaagggcaaggccaacctgactgcagtcacatctgccaccactgcctacatggagctcagcagcctgacaaatgaggaatctgcggtctattactgtacaagtacctggacccactactttgactactggggccaaggcaccactctcacagtctcctca